European Patent Specification EP 3 738 602 B1, published March 15, 2023. Title: Cell Killing Agent. Applicant: FUJITA ACADEMY. The sequence listing filed with the application follows.

SEQUENCE LISTING (5 sequences)

SEQ ID NO: 1 - protein, 19 aa, Artificial Sequence
  Description of Artificial Sequence: Effector peptide
KLAKLAKKLAKLAKHLAHL

SEQ ID NO: 2 - protein, 14 aa, Artificial Sequence
  Description of Artificial Sequence: K14D peptide
KLAKLAKKLAKLAK

SEQ ID NO: 3 - protein, 5 aa, Artificial Sequence
  Description of Artificial Sequence: H5D peptide
HLAHL

SEQ ID NO: 4 - protein, 28 aa, Artificial Sequence
  Description of Artificial Sequence: K14D-H5D-Z13 peptide
KLAKLAKKLAKLAKHLAHLVRRADNRPG

SEQ ID NO: 5 - protein, 25 aa, Artificial Sequence
  Description of Artificial Sequence: K7D-H18D peptide
KLAKLAKHLAHLAHHLAHLAHHLAH